European Patent Application EP 4 582 541 A2, published July 9, 2025. Title: FUNCTIONAL NUCLEIC ACID MOLECULE AND METHOD. Applicant: The University Court of the University of Edinburgh. The sequence listing filed with the application follows.

SEQUENCE LISTING (89 sequences)

SEQ ID NO: 1 - DNA, 15 bp, synthetic construct
  misc_feature 1..15: note = synthetic
  misc_feature 7: note = R represents A or G
  misc_feature 9: note = S represents C or G
  misc_feature 10: note = V represents A, C or G
  misc_feature 11: note = B represents C, G or T
  misc_feature 12: note = Y represents C or T
  misc_feature 14..15: note = K represents G or T
  source 1..15: mol_type = other DNA
acaaagrgsvbytkk

SEQ ID NO: 2 - DNA, 21 bp, synthetic construct
  misc_feature 1..21: note = synthetic
  misc_feature 1..4: note = R represents A or G
  misc_feature 6: note = S represents C or G
  misc_feature 8: note = R represents A or G
  misc_feature 11..13: note = R represents A or G
  misc_feature 14..15: note = B represents C, G or T
  misc_feature 16: note = H represents A
  misc_feature 17..18: note = D represents A, G or T
  misc_feature 19: note = B represents C, G or T
  misc_feature 20: note = W represents A or T
  misc_feature 21: note = H represents A, C or T
  source 1..21: mol_type = other DNA
rrrrasaragrrrbbhddbwh

SEQ ID NO: 3 - DNA, 15 bp, synthetic construct
  misc_feature 1..15: note = synthetic
  misc_feature 1: note = W represents A or T
  misc_feature 2: note = S represents C or G
  misc_feature 4: note = R represents A or G
  misc_feature 7: note = R represents A or G
  misc_feature 8: note = S represents C or G
  misc_feature 9: note = M represents A or C
  misc_feature 10: note = Y represents C or T
  misc_feature 11: note = M represents A or C
  misc_feature 12: note = H represents A, C or T
  misc_feature 14..15: note = B represents C, G or T
  source 1..15: mol_type = other DNA
wsaragrsmymhtbb

SEQ ID NO: 4 - DNA, 160 bp, synthetic construct
  misc_feature 1..160: note = synthetic
  source 1..160: mol_type = other DNA
gtgagtgtgactcacatgctggcatcagagcccctcttagagcttagaacactgggcctctgtcaggcaaagaaaaggagtccctatgaatagccatctccacaaatagcagttactgtcacttcttaaaagacacaagcatggctggagaccggcactg

SEQ ID NO: 5 - DNA, 160 bp, synthetic construct
  misc_feature 1..160: note = synthetic
  source 1..160: mol_type = other DNA
tgcatgttcttgggaaaaagtggtatttaatgaaggcgctttgagctgaatcaaagagcctcattcttctgaaagtccttcttcctagtctctgcatccggctcctatcaaaggaaatccacagctttggcttttcgttgctgttgtcatggaaatcgtt

SEQ ID NO: 6 - DNA, 160 bp, synthetic construct
  misc_feature 1..160: note = synthetic
  source 1..160: mol_type = other DNA
gaaattggatcctgaggagaatgtcaccacctctttgacaataactagctttcagagctgaacacagtgaatctggatactgtgtatatgtttaaatgagttaggaaatgacatcacattatttatttcttcttttgtgacttagtaaattgacttggcc

SEQ ID NO: 7 - DNA, 160 bp, synthetic construct
  misc_feature 1..160: note = synthetic
  source 1..160: mol_type = other DNA
tacaatctattctccatagtcatcagagtttctttaaaggcacggttcagacaatggcaccctctgttccaaaccctccagggcttcctatttcacttagcataaaaaccaaagtcctcacaatgaccgacaagtcttcacacaatgtgccccttcattg

SEQ ID NO: 8 - DNA, 160 bp, synthetic construct
  misc_feature 1..160: note = synthetic
  source 1..160: mol_type = other DNA
gagcaggcagtcatttggttcccttctctgaatgcattggctctgatccacggcgcctcaggaagtgaaagggagcaggcagtgaggccaagccatgaatgttgggcccttttcttagaaaacaaagggttcactttaggctaggaggaaacatccgggg

SEQ ID NO: 9 - DNA, 160 bp, synthetic construct
  misc_feature 1..160: note = synthetic
  source 1..160: mol_type = other DNA
gtcggcggaactgagtctcctttgtggagcccctcatttgcatgataaaccccggggacaaagtgtgttcttgttacttggactgtttcttggaaactgctgctacctggagcgagtgaacacagggcaagtattctcgcccacagcaacgtgtcattga

SEQ ID NO: 10 - DNA, 137 bp, synthetic construct
  misc_feature 1..137: note = synthetic
  source 1..137: mol_type = other DNA
caacgtttttggcagatgcagctctttctgaacagtaagtcattgttgagtgacatgaataggacgagagctacagaaaatgaaggtttcaaaagattgtctaaaacaaaagtcctttcagtcccgtattcagagtt

SEQ ID NO: 11 - DNA, 123 bp, synthetic construct
  misc_feature 1..123: note = synthetic
  source 1..123: mol_type = other DNA
ataaattccgattagccaaggaagctctgagtctaaataccagcaaagctcagcccctgcaagtggggacgaattatttgaaaggtcatcctagagacactgaacaaagggcctctagcagct

SEQ ID NO: 12 - DNA, 138 bp, synthetic construct
  misc_feature 1..138: note = synthetic
  source 1..138: mol_type = other DNA
ccaatgccaaagcagtttacattttacagatgccatggcaaccgtcaggaagttaccctgtatggtctaagagggggaggaaccctcagttccgggaattgcccgcccctttcccggaaactcatgaataatccaccc

SEQ ID NO: 13 - DNA, 161 bp, synthetic construct
  misc_feature 1..161: note = synthetic
  source 1..161: mol_type = other DNA
cgttcccccttaacaaaagccacctcctccctcctgaaaggcaccattggtcaccaaaacaagtcccctttgtcctccaccgcagctggagcctgggccttccatctcctgggggccaataaaaccccagatcagccaatcctccctccctggctctgtca

SEQ ID NO: 14 - DNA, 160 bp, synthetic construct
  misc_feature 1..160: note = synthetic
  source 1..160: mol_type = other DNA
cagcaaaggctgcacgcaatgggggagggggaaggagggaaggatatttcctcctttttagatcagtttcttttctgagcacaagtgctttctgtgtcatcctaacaatgtaagagcccactaagtttaggacgcataataccggcctttgttctactcc

SEQ ID NO: 15 - DNA, 160 bp, synthetic construct
  misc_feature 1..160: note = synthetic
  source 1..160: mol_type = other DNA
tccaaacactcccctgcaacagatgtacacacagagcccattgttttctctagaaatgtaaactgcacgtcacagttactccatacacaccacaaacagactccctttgttctcaggatatgtgttgacacaagaatatgtcatcctctcagctccagac

SEQ ID NO: 16 - DNA, 159 bp, synthetic construct
  misc_feature 1..159: note = synthetic
  source 1..159: mol_type = other DNA
tgaaagagatgggtgtgtgggagtgggggaagctgagctccaggcagacagcacagagccgccttgtccaacccagccaggtgccatggcaaccaacaaaggccccattgtcccgtgtctgctgggccttcctgaggctctggggtcagagtcccggtt

SEQ ID NO: 17 - DNA, 154 bp, synthetic construct
  misc_feature 1..154: note = synthetic
  source 1..154: mol_type = other DNA
ttgtcctgcctttgagaacactggaagggcactgaaggctgaccagcatgcacctcaccccacctcctctctgtctcatcctcagccatctaagcgggagactcatcaggcttaaattctcattcttatccaagattcttctgcttcaaatgag

SEQ ID NO: 18 - DNA, 160 bp, synthetic construct
  misc_feature 1..160: note = synthetic
  source 1..160: mol_type = other DNA
tctaaatggagatcctcccataaagggagttctgtttgggcttcccttggaagtccattgaaagcgtttcacatttcaatgcttctttacattctcctctagaatgaatctggaagggccatttcattccagccctatcagatttactacttcctcctgt

SEQ ID NO: 19 - DNA, 130 bp, synthetic construct
  misc_feature 1..130: note = synthetic
  source 1..130: mol_type = other DNA
aagaatgaactgggcccagctgggcatttgcatcaaagtgcctcaccagagttcccagctgctctggcagagtgcccaggcttgccccagagcccaaacagaatgctctttgagatgcctctggttttca

SEQ ID NO: 20 - DNA, 156 bp, synthetic construct
  misc_feature 1..156: note = synthetic
  source 1..156: mol_type = other DNA
tacccttccaggggagcagtttcctggctgtgtcgtcagatactgtggtttacgctgttccggagtctggaggtctgtgtgcctttgatctctttcccaactaatttgcacagctgctgtggaggccctcatgaatgacctctttctttcctttct

SEQ ID NO: 21 - DNA, 154 bp, synthetic construct; identical to SEQ ID NO: 17
  misc_feature 1..154: note = synthetic
  source 1..154: mol_type = other DNA

SEQ ID NO: 22 - DNA, 160 bp, synthetic construct
  misc_feature 1..160: note = synthetic
  source 1..160: mol_type = other DNA
acaaactaaacacagacattttctcaattagtcattttcaggtttattgcctaagatgctaattgaaattcagggcaggcaaaaatacatcattggcctttgtatatctttgaaaggccttctgatgggaccttgctccgtataaaggcttctcttctct

SEQ ID NO: 23 - DNA, 160 bp, synthetic construct
  misc_feature 1..160: note = synthetic
  source 1..160: mol_type = other DNA
gaccttgcctctttctggcctgtggcctttctcctcccccagctgctgtctggccgccccacccccaagtctctgccacaaccaaagctcctttgttgcctccccctgccccgggcctctccacctgctgctagctcaatcccctctttgtgtggttggt

SEQ ID NO: 24 - DNA, 160 bp, synthetic construct
  misc_feature 1..160: note = synthetic
  source 1..160: mol_type = other DNA
cattctttgcagataggaaacagtttgctatctgagagactggccaaaaaccttactttcaagtaaaatagggctctattcataagctcctacatgtacacaagttactctttatactcctttcagacaatgataagaatagaaactatttaattcagga

SEQ ID NO: 25 - DNA, 125 bp, synthetic construct
  misc_feature 1..125: note = synthetic
  source 1..125: mol_type = other DNA
acagcagccagaggaagtggctgtgtacagagagcttttgtgagagaagagggggagggggaaagagcaaagaaaaagaaggaaagaagagagggaagaggccagagacagagaaggccagagca

SEQ ID NO: 26 - DNA, 160 bp, synthetic construct
  misc_feature 1..160: note = synthetic
  source 1..160: mol_type = other DNA
atcacaaagtggttagcatgcaggggagtgcgccggtcccccgcctgtatttgcatgacaaaagcgcctgcccaacggctctcggtggctttgttgagagctgcagcctcgctcaggctgagccttgggaattgttccccgacattggttgttcctgggc

SEQ ID NO: 27 - DNA, 160 bp, synthetic construct
  misc_feature 1..160: note = synthetic
  source 1..160: mol_type = other DNA
gggcaacaaaggatgccatgcaaagcagctcagaacttgagttgtttcaacagatgctgttttatgttttgccaaagaatggccccttttatttctgtcatgaatgcagtctttctttcagtttctaaatgtttgccagtattaaccctaatccttatct

SEQ ID NO: 28 - DNA, 159 bp, synthetic construct
  misc_feature 1..159: note = synthetic
  source 1..159: mol_type = other DNA
acagaagccgttgctgcagtaaccactgccgcaagagcaactttggcagcaggcaggtgccaggcagcaagctgagagaacactgacagattcaaagtgtcttcagatacaaggctttgtttgtgcacagtgaacaaagggcatattgggaaggcctcc

SEQ ID NO: 29 - DNA, 160 bp, synthetic construct
  misc_feature 1..160: note = synthetic
  source 1..160: mol_type = other DNA
cccagactgccatctccacggcccccacaccagcacacagatgcctcattcacgtggtgctcccagggcctggcaccagttctgaggcttaaaataggcacacaacgggcctttgtcggatagaggaaggaaggaaggagcgtttcagacaaaggagaca

SEQ ID NO: 30 - DNA, 160 bp, synthetic construct
  misc_feature 1..160: note = synthetic
  source 1..160: mol_type = other DNA
accctttgcagagaggaaagagaaaggaggtctcctgttggggagatctgctttagaggttaggaagaatggtggagttgtaagacattggaatcactgtctaggaaggacagtggccttttatccagggctatttaaaaacagacagagcttcatctat

SEQ ID NO: 31 - DNA, 160 bp, synthetic construct
  misc_feature 1..160: note = synthetic
  source 1..160: mol_type = other DNA
ttcctgcatctggccctctttgagagccccttgtgtgccaatgacaaacccttctttatttaagctcctctgaagtgccttcctggtcttggcagctggacagggccctgaataagacagcgagcctcaatggcaggctaccccagggctgggtgacgta

SEQ ID NO: 32 - DNA, 159 bp, synthetic construct
  misc_feature 1..159: note = synthetic
  source 1..159: mol_type = other DNA
tgcctctcttccattggcattggagtggctataggcctttggaggacctggcaaaggggaagttgatttaggggttcattgaattgaggggaagtatgtaagtggtttgcagtcacttccttgtgtggtactcttgtatagtaatgatttcctggaata

SEQ ID NO: 33 - DNA, 150 bp, synthetic construct
  misc_feature 1..150: note = synthetic
  source 1..150: mol_type = other DNA
atgttaaacagtgaaatcatcagcaaaaagcacaaaactgcagaaaacatggcactaaatagaacacaaaaaggacacttgtttacagtatgagagcagaaacaaggaaacagtgtttccttgttcagccacagctgggaccttgtgtgt

SEQ ID NO: 34 - DNA, 105 bp, synthetic construct
  misc_feature 1..105: note = synthetic
  source 1..105: mol_type = other DNA
gcattcattttacagctggggtaagctttctctgaaatgcagctggaataggcatttcaaaggcccacagtgttatgcaaatgcttctattctccatgtgggcgg

SEQ ID NO: 35 - DNA, 85 bp, synthetic construct
  misc_feature 1..85: note = synthetic
  source 1..85: mol_type = other DNA
aaatggtgattatcatcatttgttcagggacattagcatgaaggccgaatgttctggcacaaagacacgtctgtgggacaggcac

SEQ ID NO: 36 - DNA, 130 bp, synthetic construct; identical to SEQ ID NO: 19
  misc_feature 1..130: note = synthetic
  source 1..130: mol_type = other DNA

SEQ ID NO: 37 - DNA, 890 bp, synthetic construct
  misc_feature 1..890: note = synthetic
  source 1..890: mol_type = other DNA
atctcatatatgtgtatatgtatttatgatttacatatatacagacgtatcacacactccgaatagaatacagatttccttcaatgacagcaacaactcaatgacccgcccactagcatggctaaaatactaaaccactagatagctttatgtgaacttgagcttgattgtttcttagctctgcttcagaacctcatgatcatgtgcatgcaatttctacagaagcggaaacgtagatgctgtgggtcagtgagcattcctttccagggtgcttctgagatgaagccccacgattaacacagggcccttaatgatgggcgggggactaagcattccaagattggcctggattcctgccagaagggagagaaaggggtctttgtatgtggacatctgaagggcgggcataaacatgttagttgatacttaacacccaaaaccagtgccaaaaccgttagctcccctcaatagcctactctggtttcaactgtccgcgacaatggagcagccacctcaatatacaaaacttgctctttaaacatcctcagaggaattcccaaaatagcagctgttagaagcaaacagactctaattcattgacatatgcagaccttttaatgtttttctggtgacgtttacatttttttttgtacctacgccatctatgcatttttaataattaccttgtagattacgtatgcaatccctccaggcacttgaagaaggagccccgggattcatcatcagatgaaattgttagtttttacggcaagaggcccagctaatttatgcggggaatttttcagacgtttttcctctgggctcccttccctgctgtcctcgcgcctttcttcctcagtacattaagagattctgatgtgcctgcagca

SEQ ID NO: 38 - DNA, 594 bp, synthetic construct
  misc_feature 1..594: note = synthetic
  source 1..594: mol_type = other DNA
agataaagccagaaataaaagggaaagaaacagttatatgattttggtgggaatttgcagaaatacaggctgaagctgaagtcttccatcaggtgaggttttttccattgatctcatctctcgggctcagctcttttatctccagcgcattttggatgtggcttctctttccacctgctgggcctttagatagagtacttccttttgtttcaaggtagcatttaactgagtctggaaaaaccatcattaagggaaaataaagctgaaagatgaattgaaaactatgtaaaagggccctttcaggctgccggagagattgcctttccagcctaatgagcctgtgctgcctctgattcagatggtgcaaggacaggagaaaagaatggagttttgtgcactgcgattttccaaagcacataatgcttagtcatttggggtgttaggaaagagagaaagtcggagcggagtgtgtggtgaagtgagagaaagaaagaaggctgaattttcgttaagctgctcaaatgcctgctttaacaaaagtctgccagggctagaggtgattagccatcagtgctgctgctgtttttgctgtcg

SEQ ID NO: 39 - DNA, 524 bp, synthetic construct
  misc_feature 1..524: note = synthetic
  source 1..524: mol_type = other DNA
ctctttgggtctaggtatcattttgggatcacatcatgataactctatgtgtgtgtgctgggagggcaaagttgcaaagcaattactcagcaatgctgaagaaagaagcaattactggaacacattttagccccgcttgtcagagtgactttcactggggcacaagggaagcattcacttaggcagtatccctttcagaggcttaatttagttttttcttccctttaattgtgtgattccagtattttagctacaatccctaggctgtaggaacctttaaacacttctttttataaaagaaatgcatgggcttttgaagaataaacagggggctgcataatttataggaaaatggcaccatggacttttccttcacaaagaacattggggttacattggaacaagccaaatatgtttttaatgaatagtcagtaatcagcagcagctacagtaagtgcttgaaatttttcttttatgtgctatgagtccacaaactaagcatctgattctgattgcagccatga

SEQ ID NO: 40 - DNA, 391 bp, synthetic construct
  misc_feature 1..391: note = synthetic
  source 1..391: mol_type = other DNA
gtagagaatagattctgtagggcttttaacctccactgttattccaaggatggggctcagcttccttcttttcctttctgactctgtctatatcaagggtcccgtgggttgttcctttccattgtggtctcactgcccagctttaaggcaccatcctggcacagtgataggtttacctttgtctaaaagtgtccatttgcatctctgtggccttcttgcctgggtgacacccacttgattaggcatttgcccagtgtgagatcagagtccctcatttacatttccccacaatagtgaatggcttacaggctgttcaaatacagtttctaaacagtgaataattcagccagaaagccagccttttaaggtttggatttggggcatttctgag

SEQ ID NO: 41 - DNA, 276 bp, synthetic construct
  misc_feature 1..276: note = synthetic
  source 1..276: mol_type = other DNA
tcccttggaaagtgttcaaatcaaagctacctttataccacactcctttgtgtcctgatgtcctgaatagtgagattatcgggtacacccacctgttcctgcacttccttcctgctcaatttaaataaacaatgagctgtttttcttcttgacaaagagccagtctatacaacagcagcaggaagattactttctatctgtatgcaaacagatacatagctgagttctctccaatccccgggaaaagacccttttaactaaatgacttatgcttct

SEQ ID NO: 42 - DNA, 408 bp, synthetic construct
  misc_feature 1..408: note = synthetic
  source 1..408: mol_type = other DNA
gccataatttgaacctcggagtgccccactgacagccaacgacaccagagggtccctttgtatgtaaggattgcatgactccagttgaatgacccaagccggggacaaacaggaaagaacccagcagctctggaggccacttgagctgactgtcaaatgctctgggctgattaacgactacgaacttcagggaagacaagtgtgctttgatgccacagagctatcctgggcctgtacaggcccgtttctgctctgaatgaggaagctgtactttgcaggcacccggcagaacaagaatagggcctaagatacctgaatgaagggcacagaggaagtacaaaatacagtcattgttggagctagaagctggtgccaggctacgagggggcccagtggccaagcattatg

SEQ ID NO: 43 - DNA, 345 bp, synthetic construct
  misc_feature 1..345: note = synthetic
  source 1..345: mol_type = other DNA
tgtcgggcagccaagacctgtcagggacaagagtgctgtgagctgcgggctggtgggtggaaggagagaggcccctggtgctcctgccaagccaaggaatgtgtcattgctgtgctgtgccttcagcctggcatttgggaacaaagaggtactttgtatggataacatagaccaggttgttggggaagggatcagagatgggggtagacccatttttaaaaatctgctcatgtcccaggcaagtttttttggcagggattgcagttgggctattacaaagagctgctgtacacgaggggtatgtctactactgtcaaattacagcagcaattatcttgggcactg

SEQ ID NO: 44 - DNA, 677 bp, synthetic construct
  misc_feature 1..677: note = synthetic
  source 1..677: mol_type = other DNA
ctcgatacccacattcctaaccttttaatgccaagcagcctataagcatgtcaaattttactcatgttcctgctctttccactcaagttggctttgtgggttgctggttttatcaaaattgagtgagagtgtgttcaatacaatgttggattcattagggagaaaaaagccaaataaaaaccttgcttcttcaatgccaggagcttacaaagacatataaaccatgaggaattccaaggacttgctcagaagccgttctgcaaatgcatttcttgaacaaagggccaatgttcctttcagggaagagcgcgggactggtttccggcatttttctttaaatcattaggaccatgccagcaaacaaacatatacagcccctgggagaaagaatctcattcaacacagcttacaagagtttgattattagggaggggtgcttcatggcacgtgcctcaccagccggcccccaaatgtacagatctgtttaaagggctttattgatggtggccgcagacagatagagcttgtgaggagaactgacatcccatggatactaacatatcagcatcatcctgaccagcacacaatccagtcagagagagctgaaaagtctgcctcattcccttgaaaatgtgcttcttaagacaaataaaatatagaaataagaaattcacctc

SEQ ID NO: 45 - DNA, 663 bp, synthetic construct
  misc_feature 1..663: note = synthetic
  source 1..663: mol_type = other DNA
atggacaatggcagcctgaaagaatatgagggagggtcaccagtgatggacatggtttggggagagcccaagaattgaaggggacttgggattgttgacagaccttccacatctcagaatgggggaagtggtttcttttttcctcattctccaaggcttctcagtctcagagaccccaagagatgccattaatacagattcctcctctggctcctttgagacatttgcttttgaaggacctggaagagaaagctctttgtatgtggccagaataaactcattgtacacccaaacaattaactcctcaatggacttgccagccccttgaaaggcctggccctgcgtccctggacctcttgggctctattcagtcccttaagcacaccaatgtttttgggtttttgttttgttttgtttgttattctgaaaagtctttccctgagaatagtctgagcggatcaacattgtcctcagcctggcatttatctctcctcgccagcgaatgtcaatcaggaatcaaaaagccaaacagaggaggctttgaacggtgtcatcgggggtcgaagtgacttccagctgtctgtgcgtgggccaggccttctcgcagggcaaggaattgtgctgtcacacaaacccactgtctgtataggctcacagagccca

SEQ ID NO: 46 - DNA, 365 bp, synthetic construct
  misc_feature 1..365: note = synthetic
  source 1..365: mol_type = other DNA
ctggggaacaaaacttagatcttgatcatccagcatagctctggcatgctgagcgtgtgatacacctgtctctaccgtcaggcaaacgagtgggttcacaggcagaggcctgccctgccaaacaatgctcccctttgtccccgcccagggctcaggagccgcaaggaagccaaatccatcagcacttgtcagggcccttgatgcacacaatgcaagttatgatccacagtccccggcaaagccccaggcttccagcaggcagcattaactgacacgcaatgtgtcagtcagccttctaaaagccaggggtggggatccgtgccagggggccactgagctctcattcccagaagccaaccagagcc

SEQ ID NO: 47 - DNA, 673 bp, synthetic construct
  misc_feature 1..673: note = synthetic
  source 1..673: mol_type = other DNA
gccttttagctgattaacaaatacagtgaatttaactttgtagattcttaacatttaaagacaacagtctaaggcaatttaaagtatattctgccaatcagttgttgagttagaccacccatagcctttttttattcttcattgtttgaataatatgggaggaaatttagtgtatactctcttcttcctgtattttccagttagattaagctgttgtcttcacaattgcctcccagctgctgtgacttgtgaaaacaacagaccctgctctgttgtctggagaaagccgggattgttatgagtaactttattgcaggcacatgagtgtgttaagactttaaaacacgctcaaatgtcatgtgcacacccaatgacgggcaagaataattatgaaaaaacaagaaatctatgtctatgaaaccgtgttggacaaaatgggccattcattgtgttcccctgggaatgcctggactctgcagtcagaaaacaaaaaaggcacttttttcctgccgtaggctgaatgcttagctttgccatctgagccctaagaaaacatgggcccctctactgctggcgcacccacgcacactaaaaaatattaatgcctctctctccttacttttttccaggcattccctcgtgtaggctgtagccaatataatgtcaacacaaa

SEQ ID NO: 48 - DNA, 306 bp, synthetic construct
  misc_feature 1..306: note = synthetic
  source 1..306: mol_type = other DNA
gaacagcacttaaatattaatagcatcactgggaaaacacgacagctatttccctgttttctgcagctcaatgaagagttgttcagtgcagaccccagtgctcttgcctcatgaatggacgtgattgtggggacatcatctcctactaaggcaaaacgtgacactgagaacaaaggctggtttttagcctgatgtgatgagctcaccccagtgcccatgtggggactttgaagctcgtccaggtgccagttttctgtgtatatgacattcttggttggggagggtgtggactgggcagcaggcttt

SEQ ID NO: 49 - DNA, 379 bp, synthetic construct
  misc_feature 1..379: note = synthetic
  source 1..379: mol_type = other DNA
ataagccctttaaattaaatctttatgcagattctattttatactccaaacttttcatggagccttgtgtaattctgatgtgtaaaccaacaaacagagaggctctgtgtatggagtagctggtttggataccagctggcttggctgtgcgcctttctaatggtaatgaagtcacacagctgctaggacaatcagctggagttcagattgtcactagctaaatggatatccattgactagcttcttatccggactcattaaagtttagtattgacaaatagtggctggaggtttacaactaagaggcatgtagaaatgaacttgttgactattttttccctatagcttttgctttgtgattcacagaatgtcattcatc

SEQ ID NO: 50 - DNA, 398 bp, synthetic construct
  misc_feature 1..398: note = synthetic
  source 1..398: mol_type = other DNA
gccaacaactcatatagtggaggcttgagcacaccatgcttattcccagagttccaatgctctgcttttgaaccattaccatgcctttcagcagcactgtcaacagagctcagagaaggtcttgaactccagagaatgaatgagatatgccaaatgaagcataattactttattgacgtcattcagctttcaactcacatttaatgagaaagcttctactgcttgaaacagtgggccatttgtagcacattatgcaaatgataagactaatcttttgcattatacataagagctgcttattgtgcattaactaatttatctgactaggaaggggctatgaatgctgatttttattaagctcttcattaagtgaaaatgtaggcatggcaagtgcatat

SEQ ID NO: 51 - DNA, 490 bp, synthetic construct
  misc_feature 1..490: note = synthetic
  source 1..490: mol_type = other DNA
atacattttagcaccaaacacaatttaataacagggcacagaggccgcaaagcctcctgattctgttccattactaatttatcaggggctgaaagcaaccaaacttaggatcccaggcagacaatggagcctttgaggggcaagggaagcatcatttaaaaggaaagcattaccattctaaaataatggcaaagcacatgaactgagtgctctgaaagagagcactacaaaaaaggtattctcagcttaaatgccccaaacacaaaagcttttagttgggacttagacgggaaaaagaaaatagctcccaataaattggttttaccagtatccttttgtgtgtgctggtgccaagggggcgagggtacaggcaaagcgtgattttccaaaacctagctgaattatgtttcttctttagaacaaaacccaacattttgctaatgaggataaagacagtaaaactgatattcctgtgctattactaacttgg

SEQ ID NO: 52 - DNA, 621 bp, synthetic construct
  misc_feature 1..621: note = synthetic
  source 1..621: mol_type = other DNA
cagaggagagaggaggtcatttgggaccatttactcatgcgagagtcactgccccatgctaagatttcccctaaaaataaaatgataagataataactcataatgctctccccaaatcagtaccacacagacccccctcttctgtttgctcagacccccgctctccagcacaaagtctttattggtctccctgcaggggtgaaaataaagggggttttgttcttctcctccccctcccccctcgaagggctgagtgagtttatctgacactgcagcagtctttgtaaactgagtgtcccaggataaacgctcccttaagagtcgcttggcctgggacagagggaccctctccagaggagaatggggagcttgttccaatggtcttttaatatggggggcggggtgtcaccaaggacaggcctccagcacactctcacagaagggtctctgtcctgaggctacagtggagggaattcttaaagacacagatgctgaaaagggggaaggaatttttttttcccctaaggggaggggagggaggttagggcgggaaggagaagggggagtggcgaggactcctcattccccagaacaattccagttacaacaaggcgtctctat

SEQ ID NO: 53 - DNA, 534 bp, synthetic construct
  misc_feature 1..534: note = synthetic
  source 1..534: mol_type = other DNA
aggaagaagcatgctgggtcatttttgccttgtttctagctgcatgaattgaaaagccaggcccaggttcaatgcatcattcttgaagcagtgaacaaaatccctctttgttccccagtgaaacttatctctgaagagctgcactacttcctgtgagatatagccctgcagatgtgtcgtgggagacccgcccggctgcactgccttccataaaagtgcaagaatgggcactttgtactgctggactgaaaatgacactcactcttctgatccccactggggttaccaagtgggcaaaacttcctgcttagaggaggggtcatagacagcagggggagtgtgtgattttgttttgttcctttgtgaatttgtttagctatttatagagctaaaggagaaagcaaacgggcacaatgtagcacagtgtttttcaaagtgtattccatggaaccctttcgtgggttgcagaccccaggggtggaggcagaggatggggtggtgacagcagcaggtgctgtccagggccttctgtct

SEQ ID NO: 54 - DNA, 160 bp, synthetic construct
  misc_feature 1..160: note = synthetic
  source 1..160: mol_type = other DNA
ggacaggcctccagcacactctcacagaagggtctctgtcctgaggctacagtggagggaattcttaaagacacagatgctgaaaagggggaaggaatttttttttcccctaaggggaggggagggaggttagggcgggaaggagaagggggagtggcga

SEQ ID NO: 55 - DNA, 160 bp, synthetic construct
  misc_feature 1..160: note = synthetic
  source 1..160: mol_type = other DNA
ggcaaacgagtgggttcacaggcagaggcctgccctgccaaacaatgctcccctttgtccccgcccagggctcaggagccgcaaggaagccaaatccatcagcacttgtcagggcccttgatgcacacaatgcaagttatgatccacagtccccggcaaa

SEQ ID NO: 56 - DNA, 160 bp, synthetic construct
  misc_feature 1..160: note = synthetic
  source 1..160: mol_type = other DNA
gggaagacaagtgtgctttgatgccacagagctatcctgggcctgtacaggcccgtttctgctctgaatgaggaagctgtactttgcaggcacccggcagaacaagaatagggcctaagatacctgaatgaagggcacagaggaagtacaaaatacagtc

SEQ ID NO: 57 - DNA, 160 bp, synthetic construct
  misc_feature 1..160: note = synthetic
  source 1..160: mol_type = other DNA
aatggacgtgattgtggggacatcatctcctactaaggcaaaacgtgacactgagaacaaaggctggtttttagcctgatgtgatgagctcaccccagtgcccatgtggggactttgaagctcgtccaggtgccagttttctgtgtatatgacattcttg

SEQ ID NO: 58 - DNA, 160 bp, synthetic construct
  misc_feature 1..160: note = synthetic
  source 1..160: mol_type = other DNA
caaacacaatttaataacagggcacagaggccgcaaagcctcctgattctgttccattactaatttatcaggggctgaaagcaaccaaacttaggatcccaggcagacaatggagcctttgaggggcaagggaagcatcatttaaaaggaaagcattacc

SEQ ID NO: 59 - DNA, 160 bp, synthetic construct
  misc_feature 1..160: note = synthetic
  source 1..160: mol_type = other DNA
ctccaaacttttcatggagccttgtgtaattctgatgtgtaaaccaacaaacagagaggctctgtgtatggagtagctggtttggataccagctggcttggctgtgcgcctttctaatggtaatgaagtcacacagctgctaggacaatcagctggagtt

SEQ ID NO: 60 - DNA, 160 bp, synthetic construct
  misc_feature 1..160: note = synthetic
  source 1..160: mol_type = other DNA
ggtcagtgagcattcctttccagggtgcttctgagatgaagccccacgattaacacagggcccttaatgatgggcgggggactaagcattccaagattggcctggattcctgccagaagggagagaaaggggtctttgtatgtggacatctgaagggcgg

SEQ ID NO: 61 - DNA, 160 bp, synthetic construct
  misc_feature 1..160: note = synthetic
  source 1..160: mol_type = other DNA
gatgtggcttctctttccacctgctgggcctttagatagagtacttccttttgtttcaaggtagcatttaactgagtctggaaaaaccatcattaagggaaaataaagctgaaagatgaattgaaaactatgtaaaagggccctttcaggctgccggaga

SEQ ID NO: 62 - DNA, 160 bp, synthetic construct
  misc_feature 1..160: note = synthetic
  source 1..160: mol_type = other DNA
caattactcagcaatgctgaagaaagaagcaattactggaacacattttagccccgcttgtcagagtgactttcactggggcacaagggaagcattcacttaggcagtatccctttcagaggcttaatttagttttttcttccctttaattgtgtgattc

SEQ ID NO: 63 - DNA, 160 bp, synthetic construct
  misc_feature 1..160: note = synthetic
  source 1..160: mol_type = other DNA
ttcttttcaaggatgcccaaagcgtgtgactcttacagagagccaatggggaaaggcagtgtcgggactaagcaatgaatggctcttcaatggccagctgcccgcccaataggataaaagaaaaccccacataatacttccctttgtctccaaaaaaatt

SEQ ID NO: 64 - DNA, 640 bp, synthetic construct
  misc_feature 1..640: note = synthetic
  source 1..640: mol_type = other DNA
gtgagtgtgactcacatgctggcatcagagcccctcttagagcttagaacactgggcctctgtcaggcaaagaaaaggagtccctatgaatagccatctccacaaatagcagttactgtcacttcttaaaagacacaagcatggctggagaccggcactgtgcatgttcttgggaaaaagtggtatttaatgaaggcgctttgagctgaatcaaagagcctcattcttctgaaagtccttcttcctagtctctgcatccggctcctatcaaaggaaatccacagctttggcttttcgttgctgttgtcatggaaatcgttgaaattggatcctgaggagaatgtcaccacctctttgacaataactagctttcagagctgaacacagtgaatctggatactgtgtatatgtttaaatgagttaggaaatgacatcacattatttatttcttcttttgtgacttagtaaattgacttggcctacaatctattctccatagtcatcagagtttctttaaaggcacggttcagacaatggcaccctctgttccaaaccctccagggcttcctatttcacttagcataaaaaccaaagtcctcacaatgaccgacaagtcttcacacaatgtgccccttcattg

SEQ ID NO: 65 - DNA, 640 bp, synthetic construct
  misc_feature 1..640: note = synthetic
  source 1..640: mol_type = other DNA
gaaattggatcctgaggagaatgtcaccacctctttgacaataactagctttcagagctgaacacagtgaatctggatactgtgtatatgtttaaatgagttaggaaatgacatcacattatttatttcttcttttgtgacttagtaaattgacttggcctacaatctattctccatagtcatcagagtttctttaaaggcacggttcagacaatggcaccctctgttccaaaccctccagggcttcctatttcacttagcataaaaaccaaagtcctcacaatgaccgacaagtcttcacacaatgtgccccttcattggagcaggcagtcatttggttcccttctctgaatgcattggctctgatccacggcgcctcaggaagtgaaagggagcaggcagtgaggccaagccatgaatgttgggcccttttcttagaaaacaaagggttcactttaggctaggaggaaacatccgggggtcggcggaactgagtctcctttgtggagcccctcatttgcatgataaaccccggggacaaagtgtgttcttgttacttggactgtttcttggaaactgctgctacctggagcgagtgaacacagggcaagtattctcgcccacagcaacgtgtcattga

SEQ ID NO: 66 - DNA, 580 bp, synthetic construct
  misc_feature 1..580: note = synthetic
  source 1..580: mol_type = other DNA
gagcaggcagtcatttggttcccttctctgaatgcattggctctgatccacggcgcctcaggaagtgaaagggagcaggcagtgaggccaagccatgaatgttgggcccttttcttagaaaacaaagggttcactttaggctaggaggaaacatccgggggtcggcggaactgagtctcctttgtggagcccctcatttgcatgataaaccccggggacaaagtgtgttcttgttacttggactgtttcttggaaactgctgctacctggagcgagtgaacacagggcaagtattctcgcccacagcaacgtgtcattgacaacgtttttggcagatgcagctctttctgaacagtaagtcattgttgagtgacatgaataggacgagagctacagaaaatgaaggtttcaaaagattgtctaaaacaaaagtcctttcagtcccgtattcagagttataaattccgattagccaaggaagctctgagtctaaataccagcaaagctcagcccctgcaagtggggacgaattatttgaaaggtcatcctagagacactgaacaaagggcctctagcagct

SEQ ID NO: 67 - DNA, 559 bp, synthetic construct
  misc_feature 1..559: note = synthetic
  source 1..559: mol_type = other DNA
caacgtttttggcagatgcagctctttctgaacagtaagtcattgttgagtgacatgaataggacgagagctacagaaaatgaaggtttcaaaagattgtctaaaacaaaagtcctttcagtcccgtattcagagttataaattccgattagccaaggaagctctgagtctaaataccagcaaagctcagcccctgcaagtggggacgaattatttgaaaggtcatcctagagacactgaacaaagggcctctagcagctccaatgccaaagcagtttacattttacagatgccatggcaaccgtcaggaagttaccctgtatggtctaagagggggaggaaccctcagttccgggaattgcccgcccctttcccggaaactcatgaataatccaccccgttcccccttaacaaaagccacctcctccctcctgaaaggcaccattggtcaccaaaacaagtcccctttgtcctccaccgcagctggagcctgggccttccatctcctgggggccaataaaaccccagatcagccaatcctccctccctggctctgtca

SEQ ID NO: 68 - DNA, 618 bp, synthetic construct
  misc_feature 1..618: note = synthetic
  source 1..618: mol_type = other DNA
ccaatgccaaagcagtttacattttacagatgccatggcaaccgtcaggaagttaccctgtatggtctaagagggggaggaaccctcagttccgggaattgcccgcccctttcccggaaactcatgaataatccaccccgttcccccttaacaaaagccacctcctccctcctgaaaggcaccattggtcaccaaaacaagtcccctttgtcctccaccgcagctggagcctgggccttccatctcctgggggccaataaaaccccagatcagccaatcctccctccctggctctgtcatccaaacactcccctgcaacagatgtacacacagagcccattgttttctctagaaatgtaaactgcacgtcacagttactccatacacaccacaaacagactccctttgttctcaggatatgtgttgacacaagaatatgtcatcctctcagctccagactgaaagagatgggtgtgtgggagtgggggaagctgagctccaggcagacagcacagagccgccttgtccaacccagccaggtgccatggcaaccaacaaaggccccattgtcccgtgtctgctgggccttcctgaggctctggggtcagagtcccggtt

SEQ ID NO: 69 - DNA, 633 bp, synthetic construct
  misc_feature 1..633: note = synthetic
  source 1..633: mol_type = other DNA
tccaaacactcccctgcaacagatgtacacacagagcccattgttttctctagaaatgtaaactgcacgtcacagttactccatacacaccacaaacagactccctttgttctcaggatatgtgttgacacaagaatatgtcatcctctcagctccagactgaaagagatgggtgtgtgggagtgggggaagctgagctccaggcagacagcacagagccgccttgtccaacccagccaggtgccatggcaaccaacaaaggccccattgtcccgtgtctgctgggccttcctgaggctctggggtcagagtcccggttttgtcctgcctttgagaacactggaagggcactgaaggctgaccagcatgcacctcaccccacctcctctctgtctcatcctcagccatctaagcgggagactcatcaggcttaaattctcattcttatccaagattcttctgcttcaaatgagtctaaatggagatcctcccataaagggagttctgtttgggcttcccttggaagtccattgaaagcgtttcacatttcaatgcttctttacattctcctctagaatgaatctggaagggccatttcattccagccctatcagatttactacttcctcctgt

SEQ ID NO: 70 - DNA, 600 bp, synthetic construct
  misc_feature 1..600: note = synthetic
  source 1..600: mol_type = other DNA
ttgtcctgcctttgagaacactggaagggcactgaaggctgaccagcatgcacctcaccccacctcctctctgtctcatcctcagccatctaagcgggagactcatcaggcttaaattctcattcttatccaagattcttctgcttcaaatgagtctaaatggagatcctcccataaagggagttctgtttgggcttcccttggaagtccattgaaagcgtttcacatttcaatgcttctttacattctcctctagaatgaatctggaagggccatttcattccagccctatcagatttactacttcctcctgtaagaatgaactgggcccagctgggcatttgcatcaaagtgcctcaccagagttcccagctgctctggcagagtgcccaggcttgccccagagcccaaacagaatgctctttgagatgcctctggttttcatacccttccaggggagcagtttcctggctgtgtcgtcagatactgtggtttacgctgttccggagtctggaggtctgtgtgcctttgatctctttcccaactaatttgcacagctgctgtggaggccctcatgaatgacctctttctttcctttct

SEQ ID NO: 71 - DNA, 640 bp, synthetic construct
  misc_feature 1..640: note = synthetic
  source 1..640: mol_type = other DNA
gggaagacaagtgtgctttgatgccacagagctatcctgggcctgtacaggcccgtttctgctctgaatgaggaagctgtactttgcaggcacccggcagaacaagaatagggcctaagatacctgaatgaagggcacagaggaagtacaaaatacagtcaatggacgtgattgtggggacatcatctcctactaaggcaaaacgtgacactgagaacaaaggctggtttttagcctgatgtgatgagctcaccccagtgcccatgtggggactttgaagctcgtccaggtgccagttttctgtgtatatgacattcttgctccaaacttttcatggagccttgtgtaattctgatgtgtaaaccaacaaacagagaggctctgtgtatggagtagctggtttggataccagctggcttggctgtgcgcctttctaatggtaatgaagtcacacagctgctaggacaatcagctggagttcaattactcagcaatgctgaagaaagaagcaattactggaacacattttagccccgcttgtcagagtgactttcactggggcacaagggaagcattcacttaggcagtatccctttcagaggcttaatttagttttttcttccctttaattgtgtgattc

SEQ ID NO: 72 - DNA, 640 bp, synthetic construct
  misc_feature 1..640: note = synthetic
  source 1..640: mol_type = other DNA
gggaagacaagtgtgctttgatgccacagagctatcctgggcctgtacaggcccgtttctgctctgaatgaggaagctgtactttgcaggcacccggcagaacaagaatagggcctaagatacctgaatgaagggcacagaggaagtacaaaatacagtccaaacacaatttaataacagggcacagaggccgcaaagcctcctgattctgttccattactaatttatcaggggctgaaagcaaccaaacttaggatcccaggcagacaatggagcctttgaggggcaagggaagcatcatttaaaaggaaagcattaccctccaaacttttcatggagccttgtgtaattctgatgtgtaaaccaacaaacagagaggctctgtgtatggagtagctggtttggataccagctggcttggctgtgcgcctttctaatggtaatgaagtcacacagctgctaggacaatcagctggagttcaattactcagcaatgctgaagaaagaagcaattactggaacacattttagccccgcttgtcagagtgactttcactggggcacaagggaagcattcacttaggcagtatccctttcagaggcttaatttagttttttcttccctttaattgtgtgattc

SEQ ID NO: 73 - DNA, 640 bp, synthetic construct
  misc_feature 1..640: note = synthetic
  source 1..640: mol_type = other DNA
aatggacgtgattgtggggacatcatctcctactaaggcaaaacgtgacactgagaacaaaggctggtttttagcctgatgtgatgagctcaccccagtgcccatgtggggactttgaagctcgtccaggtgccagttttctgtgtatatgacattcttgcaaacacaatttaataacagggcacagaggccgcaaagcctcctgattctgttccattactaatttatcaggggctgaaagcaaccaaacttaggatcccaggcagacaatggagcctttgaggggcaagggaagcatcatttaaaaggaaagcattaccggtcagtgagcattcctttccagggtgcttctgagatgaagccccacgattaacacagggcccttaatgatgggcgggggactaagcattccaagattggcctggattcctgccagaagggagagaaaggggtctttgtatgtggacatctgaagggcggcaattactcagcaatgctgaagaaagaagcaattactggaacacattttagccccgcttgtcagagtgactttcactggggcacaagggaagcattcacttaggcagtatccctttcagaggcttaatttagttttttcttccctttaattgtgtgattc

SEQ ID NO: 74 - DNA, 640 bp, synthetic construct
  misc_feature 1..640: note = synthetic
  source 1..640: mol_type = other DNA
ctccaaacttttcatggagccttgtgtaattctgatgtgtaaaccaacaaacagagaggctctgtgtatggagtagctggtttggataccagctggcttggctgtgcgcctttctaatggtaatgaagtcacacagctgctaggacaatcagctggagttggtcagtgagcattcctttccagggtgcttctgagatgaagccccacgattaacacagggcccttaatgatgggcgggggactaagcattccaagattggcctggattcctgccagaagggagagaaaggggtctttgtatgtggacatctgaagggcggcaattactcagcaatgctgaagaaagaagcaattactggaacacattttagccccgcttgtcagagtgactttcactggggcacaagggaagcattcacttaggcagtatccctttcagaggcttaatttagttttttcttccctttaattgtgtgattcttcttttcaaggatgcccaaagcgtgtgactcttacagagagccaatggggaaaggcagtgtcgggactaagcaatgaatggctcttcaatggccagctgcccgcccaataggataaaagaaaaccccacataatacttccctttgtctccaaaaaaatt

SEQ ID NO: 75 - DNA, 640 bp, synthetic construct
  misc_feature 1..640: note = synthetic
  source 1..640: mol_type = other DNA
gggaagacaagtgtgctttgatgccacagagctatcctgggcctgtacaggcccgtttctgctctgaatgaggaagctgtactttgcaggcacccggcagaacaagaatagggcctaagatacctgaatgaagggcacagaggaagtacaaaatacagtcctccaaacttttcatggagccttgtgtaattctgatgtgtaaaccaacaaacagagaggctctgtgtatggagtagctggtttggataccagctggcttggctgtgcgcctttctaatggtaatgaagtcacacagctgctaggacaatcagctggagttggtcagtgagcattcctttccagggtgcttctgagatgaagccccacgattaacacagggcccttaatgatgggcgggggactaagcattccaagattggcctggattcctgccagaagggagagaaaggggtctttgtatgtggacatctgaagggcggcaattactcagcaatgctgaagaaagaagcaattactggaacacattttagccccgcttgtcagagtgactttcactggggcacaagggaagcattcacttaggcagtatccctttcagaggcttaatttagttttttcttccctttaattgtgtgattc

SEQ ID NO: 76 - DNA, 640 bp, synthetic construct
  misc_feature 1..640: note = synthetic
  source 1..640: mol_type = other DNA
caaacacaatttaataacagggcacagaggccgcaaagcctcctgattctgttccattactaatttatcaggggctgaaagcaaccaaacttaggatcccaggcagacaatggagcctttgaggggcaagggaagcatcatttaaaaggaaagcattaccctccaaacttttcatggagccttgtgtaattctgatgtgtaaaccaacaaacagagaggctctgtgtatggagtagctggtttggataccagctggcttggctgtgcgcctttctaatggtaatgaagtcacacagctgctaggacaatcagctggagttggtcagtgagcattcctttccagggtgcttctgagatgaagccccacgattaacacagggcccttaatgatgggcgggggactaagcattccaagattggcctggattcctgccagaagggagagaaaggggtctttgtatgtggacatctgaagggcggttcttttcaaggatgcccaaagcgtgtgactcttacagagagccaatggggaaaggcagtgtcgggactaagcaatgaatggctcttcaatggccagctgcccgcccaataggataaaagaaaaccccacataatacttccctttgtctccaaaaaaatt

SEQ ID NO: 77 - DNA, 640 bp, synthetic construct
  misc_feature 1..640: note = synthetic
  source 1..640: mol_type = other DNA
gggaagacaagtgtgctttgatgccacagagctatcctgggcctgtacaggcccgtttctgctctgaatgaggaagctgtactttgcaggcacccggcagaacaagaatagggcctaagatacctgaatgaagggcacagaggaagtacaaaatacagtcaatggacgtgattgtggggacatcatctcctactaaggcaaaacgtgacactgagaacaaaggctggtttttagcctgatgtgatgagctcaccccagtgcccatgtggggactttgaagctcgtccaggtgccagttttctgtgtatatgacattcttgcaattactcagcaatgctgaagaaagaagcaattactggaacacattttagccccgcttgtcagagtgactttcactggggcacaagggaagcattcacttaggcagtatccctttcagaggcttaatttagttttttcttccctttaattgtgtgattcttcttttcaaggatgcccaaagcgtgtgactcttacagagagccaatggggaaaggcagtgtcgggactaagcaatgaatggctcttcaatggccagctgcccgcccaataggataaaagaaaaccccacataatacttccctttgtctccaaaaaaatt

SEQ ID NO: 78 - DNA, 640 bp, synthetic construct
  misc_feature 1..640: note = synthetic
  source 1..640: mol_type = other DNA
gggaagacaagtgtgctttgatgccacagagctatcctgggcctgtacaggcccgtttctgctctgaatgaggaagctgtactttgcaggcacccggcagaacaagaatagggcctaagatacctgaatgaagggcacagaggaagtacaaaatacagtcaatggacgtgattgtggggacatcatctcctactaaggcaaaacgtgacactgagaacaaaggctggtttttagcctgatgtgatgagctcaccccagtgcccatgtggggactttgaagctcgtccaggtgccagttttctgtgtatatgacattcttgctccaaacttttcatggagccttgtgtaattctgatgtgtaaaccaacaaacagagaggctctgtgtatggagtagctggtttggataccagctggcttggctgtgcgcctttctaatggtaatgaagtcacacagctgctaggacaatcagctggagttttcttttcaaggatgcccaaagcgtgtgactcttacagagagccaatggggaaaggcagtgtcgggactaagcaatgaatggctcttcaatggccagctgcccgcccaataggataaaagaaaaccccacataatacttccctttgtctccaaaaaaatt

SEQ ID NO: 79 - DNA, 640 bp, synthetic construct
  misc_feature 1..640: note = synthetic
  source 1..640: mol_type = other DNA
ctccaaacttttcatggagccttgtgtaattctgatgtgtaaaccaacaaacagagaggctctgtgtatggagtagctggtttggataccagctggcttggctgtgcgcctttctaatggtaatgaagtcacacagctgctaggacaatcagctggagttggtcagtgagcattcctttccagggtgcttctgagatgaagccccacgattaacacagggcccttaatgatgggcgggggactaagcattccaagattggcctggattcctgccagaagggagagaaaggggtctttgtatgtggacatctgaagggcgggatgtggcttctctttccacctgctgggcctttagatagagtacttccttttgtttcaaggtagcatttaactgagtctggaaaaaccatcattaagggaaaataaagctgaaagatgaattgaaaactatgtaaaagggccctttcaggctgccggagacaattactcagcaatgctgaagaaagaagcaattactggaacacattttagccccgcttgtcagagtgactttcactggggcacaagggaagcattcacttaggcagtatccctttcagaggcttaatttagttttttcttccctttaattgtgtgattc

SEQ ID NO: 80 - DNA, 640 bp, synthetic construct
  misc_feature 1..640: note = synthetic
  source 1..640: mol_type = other DNA
caaacacaatttaataacagggcacagaggccgcaaagcctcctgattctgttccattactaatttatcaggggctgaaagcaaccaaacttagggcagacaatggagcctttgaggggcaagggaagcatcatttaaaaggaaagcattaccggtcagtgagcattcctttccagggtgcttctgagatgaagccccacgattaacacagggcccttaatgatgggcgggggactaagcattccaagattggcctggattcctgccagaagggagagaaaggggtctttgtatgtggacatctgaagggcggcaattactcagcaatgctgaagaaagaagcaattactggaacacattttagccccgcttgtcagagtgactttcactggggcacaagggaagcattcacttaggcagtatccctttcagaggcttaatttagttttttcttccctttaattgtgtgattcttcttttcaaggatgcccaaagcgtgtgactcttacagagagccaatggggaaaggcagtgtcgggactaagcaatgaatggctcttcaatggccagctgcccgcccaataggataaaagaaaaccccacataatacttccctttgtctccaaaaaaattatcccag

SEQ ID NO: 81 - DNA, 36 bp, synthetic construct
  misc_feature 1..36: note = synthetic
  source 1..36: mol_type = other DNA
tgatccgtctcgccctactaggttactggtgcatgc

SEQ ID NO: 82 - DNA, 36 bp, synthetic construct
  misc_feature 1..36: note = synthetic
  source 1..36: mol_type = other DNA
actaacgtctcggagcacccaaactattggagcgag

SEQ ID NO: 83 - DNA, 15 bp, synthetic construct
  misc_feature 1..15: note = synthetic
  source 1..15: mol_type = other DNA
tcaaagagcctcatt

SEQ ID NO: 84 - DNA, 13 bp, synthetic construct
  misc_feature 1..13: note = synthetic
  source 1..13: mol_type = other DNA
tcaaagagccatt

SEQ ID NO: 85 - DNA, 17 bp, synthetic construct
  misc_feature 1..17: note = synthetic
  source 1..17: mol_type = other DNA
tcaaagagatcctcatt

SEQ ID NO: 86 - DNA, 15 bp, synthetic construct
  misc_feature 1..15: note = synthetic
  source 1..15: mol_type = other DNA
ttactccgagaaact

SEQ ID NO: 87 - DNA, 15 bp, synthetic construct
  misc_feature 1..15: note = synthetic
  source 1..15: mol_type = other DNA
tctaagagcctcaat

SEQ ID NO: 88 - DNA, 16 bp, synthetic construct
  misc_feature 1..16: note = synthetic
  source 1..16: mol_type = other DNA
aacaatatgcagtgtt

SEQ ID NO: 89 - DNA, 15 bp, synthetic construct
  misc_feature 1..15: note = synthetic
  source 1..15: mol_type = other DNA
ggcgatatcgtacgc